European Patent Application EP 4 279 583 A2, published November 22, 2023. Title: DIFFERENTIATION OF PLURIPOTENT STEM CELLS TO FORM RENAL ORGANOIDS. Applicant: The University of Queensland. Application EP. The sequence listing filed with the application follows.

SEQUENCE LISTING (14 sequences)

SEQ ID NO: 1 - DNA, 19 bp, synthetic construct
  misc_feature 1..19: note = Forward primer T
  source 1..19: mol_type = other DNA
aggtacccaaccctgagga

SEQ ID NO: 2 - DNA, 23 bp, synthetic construct
  misc_feature 1..23: note = Reverse primer T
  source 1..23: mol_type = other DNA
gcaggtgagttgtcagaataggt

SEQ ID NO: 3 - DNA, 20 bp, synthetic construct
  misc_feature 1..20: note = Forward primer LHX1
  source 1..20: mol_type = other DNA
atgcaacctgaccgagaagt

SEQ ID NO: 4 - DNA, 19 bp, synthetic construct
  misc_feature 1..19: note = Reverse primer LHX1
  source 1..19: mol_type = other DNA
caggtcgctaggggagatg

SEQ ID NO: 5 - DNA, 21 bp, synthetic construct
  misc_feature 1..21: note = Forward primer TBX6
  source 1..21: mol_type = other DNA
catccacgagaattgtacccg

SEQ ID NO: 6 - DNA, 21 bp, synthetic construct
  misc_feature 1..21: note = Reverse primer TBX6
  source 1..21: mol_type = other DNA
agcaatccagtttaggggtgt

SEQ ID NO: 7 - DNA, 19 bp, synthetic construct
  misc_feature 1..19: note = Forward primer GATA3
  source 1..19: mol_type = other DNA
gcccctcattaagcccaag

SEQ ID NO: 8 - DNA, 21 bp, synthetic construct
  misc_feature 1..21: note = Reverse primer GATA3
  source 1..21: mol_type = other DNA
ttgtggtggtctgacagttcg

SEQ ID NO: 9 - DNA, 20 bp, synthetic construct
  misc_feature 1..20: note = Forward primer HOXD11
  source 1..20: mol_type = other DNA
gccagtgtgctgtcgttccc

SEQ ID NO: 10 - DNA, 20 bp, synthetic construct
  misc_feature 1..20: note = Reverse primer HOXD11
  source 1..20: mol_type = other DNA
cttcctacagaccccgccgt

SEQ ID NO: 11 - DNA, 20 bp, synthetic construct
  misc_feature 1..20: note = Forward primer EYA1
  source 1..20: mol_type = other DNA
atctaaccagcccgcatagc

SEQ ID NO: 12 - DNA, 20 bp, synthetic construct
  misc_feature 1..20: note = Reverse primer EYA1
  source 1..20: mol_type = other DNA
gtgccattgggagtcatgga

SEQ ID NO: 13 - DNA, 19 bp, synthetic construct
  misc_feature 1..19: note = Forward primer GAPDH
  source 1..19: mol_type = other DNA
agccacatcgctcagacac

SEQ ID NO: 14 - DNA, 19 bp, synthetic construct
  misc_feature 1..19: note = Reverse primer GAPDH
  source 1..19: mol_type = other DNA
gcccaatacgaccaaatcc